European Patent Specification EP 3 796 933 B1, published September 23, 2026. Title: Methods for Treating, Preventing and Detecting the Prognosis of Colorectal Cancer. Applicant: The Trustees of Columbia University in the City of New York. Application Filed Herewith. The sequence listing filed with the application follows.

SEQUENCE LISTING (26 sequences)

SEQ ID NO: 1 - RNA, 25 nt, Artificial Sequence
  Synthetic siRNA
uaaccauuauggccuuaugcaaggc

SEQ ID NO: 2 - RNA, 25 nt, Artificial Sequence
  Synthetic siRNA
uuaaucuccagccaguuggcagugu

SEQ ID NO: 3 - DNA, 20 bp, Artificial Sequence
  Synthetic Primer
gcaggcctggtttattgaaa

SEQ ID NO: 4 - DNA, 20 bp, Artificial Sequence
  Synthetic Primer
gctgtgcattgtttcgctta

SEQ ID NO: 5 - DNA, 23 bp, Artificial Sequence
  Synthetic Primer
tagcacaaaatgaacaagtttac

SEQ ID NO: 6 - DNA, 21 bp, Artificial Sequence
  Synthetic Primer
ataaaatcttgtgttagcttc

SEQ ID NO: 7 - DNA, 20 bp, Artificial Sequence
  Synthetic Primer
actcctacgggaggcagcag

SEQ ID NO: 8 - DNA, 17 bp, Artificial Sequence
  Synthetic Primer
attaccgcggctgctgg

SEQ ID NO: 9 - DNA, 25 bp, Artificial Sequence
  Synthetic Primer
caaccatcattgacattcttaccaa

SEQ ID NO: 10 - DNA, 19 bp, Artificial Sequence
  Synthetic Primer
tggcaccacggagttcatc

SEQ ID NO: 11 - DNA, 25 bp, Artificial Sequence
  Synthetic Primer
aaacagatgaagtgctccttccagg

SEQ ID NO: 12 - DNA, 24 bp, Artificial Sequence
  Synthetic Primer
tggagaacaccacttgttgctcca

SEQ ID NO: 13 - DNA, 21 bp, Artificial Sequence
  Synthetic Primer
ggagcaagaggccaaagaact

SEQ ID NO: 14 - DNA, 21 bp, Artificial Sequence
  Synthetic Primer
tacaggccgctcaatcttcat

SEQ ID NO: 15 - DNA, 22 bp, Artificial Sequence
  Synthetic Primer
gctgtcatcctcattgctactg

SEQ ID NO: 16 - DNA, 25 bp, Artificial Sequence
  Synthetic Primer
tggtgtagaaatactccttgatgtg

SEQ ID NO: 17 - DNA, 20 bp, Artificial Sequence
  Synthetic Primer
ctggctgctttgatgtcagt

SEQ ID NO: 18 - DNA, 20 bp, Artificial Sequence
  Synthetic Primer
cgtgtgaagcccacaataaa

SEQ ID NO: 19 - DNA, 21 bp, Artificial Sequence
  Synthetic Primer
acaaactgttttgaaaatcca

SEQ ID NO: 20 - DNA, 20 bp, Artificial Sequence
  Synthetic Primer
cgagtcattgcatactgtcc

SEQ ID NO: 21 - DNA, 20 bp, Artificial Sequence
  Synthetic Primer
agccagatcactgctgaggt

SEQ ID NO: 22 - DNA, 20 bp, Artificial Sequence
  Synthetic Primer
tggacaggtgttcctccttc

SEQ ID NO: 23 - DNA, 25 bp, Artificial Sequence
  Synthetic Primer
aatccaaagcctcaggtcataaaca

SEQ ID NO: 24 - DNA, 24 bp, Artificial Sequence
  Synthetic Primer
ggttgggtcgttgtactgaatggt

SEQ ID NO: 25 - DNA, 25 bp, Artificial Sequence
  Synthetic Primer
tcaaaaatggcaatggtatcagaat

SEQ ID NO: 26 - DNA, 20 bp, Artificial Sequence
  Synthetic Primer
gtttcctccacaaagagcca